European Patent Application EP 4 745 574 A1, published May 20, 2026. Title: 联合检测抗MCV抗体、抗CCP抗体和RF的荧光免疫层析试纸条. Applicant: 深圳市睿盟创新生物科技有限公司. The sequence listing filed with the application follows.

SEQUENCE LISTING (2 sequences)

SEQ ID NO: 1 - protein, 473 aa, synthetic construct
  SITE 4: note = X is Citrulline
  SITE 17: note = X is Citrulline
  SITE 28: note = X is Citrulline
  SITE 41: note = X is Citrulline
  SITE 50: note = X is Citrulline
  SITE 69: note = X is Citrulline
  SITE 76: note = X is Citrulline
  SITE 145: note = X is Citrulline
  SITE 159: note = X is Citrulline
  SITE 184: note = X is Citrulline
  SITE 217: note = X is Citrulline
  SITE 440: note = X is Citrulline
  SITE 462: note = X is Citrulline
MSTXSVSSSSYRGMFGXPGTASGPSSSXSYVTTSTRTYSLXSALGPSTSXSLYASSPGRVYATGSSYVXLRSSVPXVGLLQDSVDFSLADAINTEFKNTRTNEKVELQELNDRFANYIDKVRFLEQQNKILLAELEQLKGQGKSXLGDLYEEEMRELRXQVDQLTNDKARVEVERDNLAEDIMXLREKLQEEMLQREEAENTLQSFRQDVDNASLAXLDLERKVESLQEEIAFLKKLHEEEIQELQAQIQEQHVQIDVDVSKPDLTAALRDVRQQYESVAAKNLQEAEEWYKSKFADLSEAANRNNDALRQAKQESTEYRRQVQSLTCEVDALKGTNESLERQMREMEENFAVEAANYQDTIGGLQDEIQNMKEEMAGHLREYQDLLNVKMALDIEIATYGKLLEGEESRISLPLPNFSSLNLGETNLDSLPLVDTHSKXTLLIKTVETRDRQVINETSQHXDDLEGHHHHHH

SEQ ID NO: 2 - protein, 21 aa, synthetic construct
  SITE 10: note = X is Citrulline
HQCHQSSTGXHRHGRCGRTGS